European Patent Application EP 4 527 924 A2, published March 26, 2025. Title: Method for optimizing mRNA sequence using peptide barcodes. Applicant: Hitachi, Ltd. The sequence listing filed with the application follows.

SEQUENCE LISTING (9 sequences)

SEQ ID NO: 1 - protein, 5 aa, synthetic construct
  REGION 1..5: note = synthetic peptide
DDDDK

SEQ ID NO: 2 - DNA, 59 bp, synthetic construct
  misc_feature 1..59: note = synthetic polynucleotide
  source 1..59: mol_type = other DNA
agagcggaggtggtggcggcggaggctttggcagctcgggactgagtgcaagaatcagc

SEQ ID NO: 3 - DNA, 140 bp, synthetic construct
  misc_feature 1..140: note = synthetic polynucleotide
  source 1..140: mol_type = other DNA
agaaataaagtaaaattaatctggtaatttgtcacggattagttgtacaactagttagaagtttcagaataaacatgcatttcataactgtcaaatgttcttttaattctgagtccaaataaattatttggtgatgttga

SEQ ID NO: 4 - DNA, 37 bp, synthetic construct
  misc_feature 1..37: note = synthetic polynucleotide
  source 1..37: mol_type = other DNA
actcttctggtccccacagactcagagagaacccacc

SEQ ID NO: 5 - DNA, 109 bp, synthetic construct
  misc_feature 1..109: note = synthetic polynucleotide
  source 1..109: mol_type = other DNA
gctggagcctcggtagccgttcctcctgcccgctgggcctcccaacgggccctcctcccctccttgcaccggcccttcctggtctttgaataaagtctgagtgggcagc

SEQ ID NO: 6 - protein, 14 aa, synthetic construct
  REGION 1..14: note = synthetic peptide
FVGARLDYKDDDDK

SEQ ID NO: 7 - DNA, 75 bp, synthetic construct
  misc_feature 1..75: note = synthetic polynucleotide
  source 1..75: mol_type = other DNA
ggcggtagtgactacaaagatgacgacgataaatttgtcggtgcccgtctagactacaaggatgatgatgacaag

SEQ ID NO: 8 - protein, 14 aa, synthetic construct
  REGION 1..14: note = synthetic peptide
WLFPVGDYKDDDDK

SEQ ID NO: 9 - DNA, 75 bp, synthetic construct
  misc_feature 1..75: note = synthetic polynucleotide
  source 1..75: mol_type = other DNA
ggaggcagtgactacaaagatgacgacgataaatggctgttccctgtcggagactataaggatgatgatgataag